European Patent Specification EP 3 541 409 B1, published January 22, 2025. Title: ENGINEERED TGF-BETA MONOMERS AND THEIR USE FOR INHIBITING TGF-BETA SIGNALING. Applicant: UNIVERSITY OF PITTSBURGH - OF THE COMMONWEALTH SYSTEM OF HIGHER EDUCATION THE BOARD OF REGENTS OF THE UNIVERSITY OF TEXAS SYSTEM NATIONAL RESEARCH COUNCIL OF CANADA. The sequence listing filed with the application follows.

SEQUENCE LISTING (11 sequences)

SEQ ID NO: 1 - protein, 113 aa, Homo sapiens
MALDTNYCFSSTEKNCCVRQLYIDFRKDLGWKWIHEPKGYHANFCLGPCPYIWSLDTQYSKVLALYNQHNPGASAAPCCVPQALEPLPIVYYVGRKPKVEQLSNMIVRSCKCS

SEQ ID NO: 2 - protein, 113 aa, Homo sapiens
MALDAAYCFRNVQDNCCLRPLYIDFKRDLGWKWIHEPKGYNANFCAGACPYLWSSDTQHSKVLSLYNTINPEASASPCCVSQDLEPLTILYYIGKTPKIEQLSNMIVKSCKCS

SEQ ID NO: 3 - protein, 113 aa, Homo sapiens
MALDTNYCFRNLEENCCVRPLYIDFRQDLGWKWVHEPKGYYANFCSGPCPYLRSADTTHSTVLGLYNTLNPEASASPCCVPQDLEPLTILYYVGRTPKVEQLSNMVVKSCKCS

SEQ ID NO: 4 - protein, 130 aa, Artificial Sequence
  Synthetic polypeptide
MGLNDIFEAQKIEWHEEFALDTNYCFRNLEENCCVRPLYIDFRQDLGWKWVHEPKGYYANFCSGPCPYLRSADTTHSTVLGLYNTLNPEASASPCCVPQDLEPLTILYYVGRTPKVEQLSNMVVKSCKCS

SEQ ID NO: 5 - protein, 113 aa, Artificial Sequence
  Synthetic polypeptide
MALDAAYCFRNVQDNCCLRPLYIDFKRDLGWKWIHEPKGYNANFCAGACPYLWSSDTQHSKVLSLYNTINPEASASPSCVSQDLEPLTILYYIGKTPKIEQLSNMIVKSCKCS

SEQ ID NO: 6 - protein, 113 aa, Artificial Sequence
  Synthetic polypeptide
MALDTNYCFRNLEENCCVRPLYIDFRQDLGWKWVHEPKGYYANFCSGPCPYLRSADTTHSTVLGLYNTLNPEASASPSCVPQDLEPLTILYYVGRTPKVEQLSNMVVKSCKCS

SEQ ID NO: 7 - protein, 93 aa, Artificial Sequence
  Synthetic polypeptide
MALDTNYCFSSTEKNCCVRQLYIDFRKDLGWKWIHEPKGYHANFCLGPCPYRASKSPSCVPQALEPLPIVYYVGRKPKVEQLSNMIVRSCKCS

SEQ ID NO: 8 - protein, 93 aa, Artificial Sequence
  Synthetic polypeptide
MALDAAYCFRNVQDNCCLRPLYIDFKRDLGWKWIHEPKGYNANFCAGACPYRASKSPSCVSQDLEPLTILYYIGKTPKIEQLSNMIVKSCKCS

SEQ ID NO: 9 - protein, 93 aa, Artificial Sequence
  Synthetic polypeptide
MALDTNYCFRNLEENCCVRPLYIDFRQDLGWKWVHEPKGYYANFCSGPCPYEESDSPSCVPQDLEPLTILYYVGRTPKVEQLSNMVVKSCKCS

SEQ ID NO: 10 - protein, 93 aa, Artificial Sequence
  Synthetic polypeptide
MALDAAYCFRNVQDNCCLRPLYIDFRKDLGWKWIHEPKGYNANFCAGACPYRASKSPSCVSQDLEPLTIVYYVGRKPKVEQLSNMIVKSCKCS

SEQ ID NO: 11 - protein, 110 aa, Artificial Sequence
  Synthetic polypeptide
MGLNDIFEAQKIEWHEEFALDAAYCFRNVQDNCCLRPLYIDFRKDLGWKWIHEPKGYNANFCAGACPYRASKSPSCVSQDLEPLTIVYYVGRKPKVEQLSNMIVKSCKCS